European Patent Specification EP 3 325 631 B1, published September 3, 2025. Title: Rekombinanter Orf-Virus-Vektor. Applicant: Eberhard Karls Universität. The sequence listing filed with the application follows.

SEQUENCE LISTING (5 sequences)

SEQ ID NO: 1 - DNA, 16 bp, Künstliche Sequenz
  Promotor
aaaaattgaaaaatta

SEQ ID NO: 2 - DNA, 16 bp, Künstliche Sequenz
  Promotor
aaaaattgaaattcta

SEQ ID NO: 3 - DNA, 16 bp, Künstliche Sequenz
  Promotor
aaaaattgaaaaayta

SEQ ID NO: 4 - DNA, 15 bp, Künstliche Sequenz
  Promotor
aaaagtagaaaatta

SEQ ID NO: 5 - DNA, 16 bp, Künstliche Sequenz
  VEGF
caaaatgtaaattata